European Patent Specification EP 3 318 275 B1, published April 2, 2025. Title: Novel sepsis treating agent and/or method for screening thereof. Applicant: Tadamitsu, Kishimoto Kazuya, Masuda CHUGAI SEIYAKU KABUSHIKI KAISHA. The sequence listing filed with the application follows.

SEQUENCE LISTING (2 sequences)

SEQ ID NO: 1 - DNA, 20 bp, Artificial Sequence
  primer1
atactttctcggcaggagca

SEQ ID NO: 2 - DNA, 20 bp, Artificial Sequence
  primer2
tgaatgaactgcaggacgag